European Patent Specification EP 3 665 190 B1, published July 26, 2023. Title: DISINTEGRIN VARIANTS AND USES THEREOF. Applicant: NATIONAL TAIWAN UNIVERSITY NATIONAL CHENG KUNG UNIVERSITY DCB-USA LLC. The sequence listing filed with the application follows.

SEQUENCE LISTING (25 sequences)

SEQ ID NO: 1 - protein, 5 aa, Artificial Sequence
  TMV-7_Linker region
KKKRT

SEQ ID NO: 2 - protein, 6 aa, Artificial Sequence
  TMV-7_RGD region
ARGDNP

SEQ ID NO: 3 - protein, 7 aa, Artificial Sequence
  TMV-7_C-terminus
PRNGLYG

SEQ ID NO: 4 - protein, 5 aa, Artificial Sequence
  Rhodostomin_Linker region
SRAGK

SEQ ID NO: 5 - protein, 6 aa, Artificial Sequence
  Rhodostomin_RGD region
PRGDMP

SEQ ID NO: 6 - protein, 4 aa, Artificial Sequence
  Rhodostomin_C-terminus
PRYH

SEQ ID NO: 7 - protein, 5 aa, Artificial Sequence
  T/IEEGKRR_Linker region
IEEGT

SEQ ID NO: 8 - protein, 5 aa, Artificial Sequence
  T/AKRRR_Linker region
KKART

SEQ ID NO: 9 - protein, 5 aa, Artificial Sequence
  T/MGKRRR_Linker region
MKKGT

SEQ ID NO: 10 - protein, 6 aa, Artificial Sequence
  T/KH_RGD region
AKGDHP

SEQ ID NO: 11 - protein, 6 aa, Artificial Sequence
  T/KY_RGD region
AKGDYP

SEQ ID NO: 12 - protein, 6 aa, Artificial Sequence
  T/KWR_RGD region
AKGDWP

SEQ ID NO: 13 - protein, 6 aa, Artificial Sequence
  T/KRR_RGD region
AKGDRP

SEQ ID NO: 14 - protein, 6 aa, Artificial Sequence
  T/KRRR_RGD region
AKGDRR

SEQ ID NO: 15 - protein, 6 aa, Artificial Sequence
  T/KRKR_RGD region
AKGDRK

SEQ ID NO: 16 - protein, 6 aa, Artificial Sequence
  T/KKRR_RGD region
AKGDKR

SEQ ID NO: 17 - protein, 6 aa, Artificial Sequence
  T/KKKR_RGD region
AKGDKK

SEQ ID NO: 18 - protein, 6 aa, Artificial Sequence
  T/K_RGD region
AKGDNP

SEQ ID NO: 19 - protein, 6 aa, Artificial Sequence
  T/KF_RGD region
AKGDFP

SEQ ID NO: 20 - protein, 6 aa, Artificial Sequence
  T/KWN_RGD region
AKGDWN

SEQ ID NO: 21 - protein, 7 aa, Artificial Sequence
  T/KHR_C-terminus
PRNRLYG

SEQ ID NO: 22 - protein, 4 aa, Artificial Sequence
  T/KS_C terminus
PRNS

SEQ ID NO: 23 - protein, 6 aa, Artificial Sequence
  T/KRRFH_C terminus
PRNRFH

SEQ ID NO: 24 - protein, 6 aa, Artificial Sequence
  R/K_RGD region
PKGDMP

SEQ ID NO: 25 - protein, 6 aa, Artificial Sequence
  R/AWN_RGD region
ARGDWN